European Patent Specification EP 4 274 802 B1, published July 15, 2026. Title: MODULAR KINETICALLY-CONTROLLED FUNCTIONAL RNA CONSTRUCTS AND RELATED COMPOSITIONS, SYSTEMS, AND METHODS. Applicant: University of Washington. The sequence listing filed with the application follows.

SEQUENCE LISTING (49 sequences)

SEQ ID NO: 1 - DNA, 30 bp, Artificial sequence
  Synthetic
ctttttgagatcgaaattctaagtagaaag

SEQ ID NO: 2 - DNA, 30 bp, Artificial sequence
  Synthetic
gtttaggaaattgaaaggttaagtctaaaa

SEQ ID NO: 3 - DNA, 30 bp, Artificial sequence
  Synthetic
atttacgaacaggaaaggtaaagtgtaaat

SEQ ID NO: 4 - DNA, 30 bp, Artificial sequence
  Synthetic
tttttcgatctggaaaaggaaagtggaaag

SEQ ID NO: 5 - DNA, 30 bp, Artificial sequence
  Synthetic
ctttatgagggtgaaatcctaagtgtaaat

SEQ ID NO: 6 - DNA, 30 bp, Artificial sequence
  Synthetic
atttaggattaagaaattttaagtctaaag

SEQ ID NO: 7 - DNA, 30 bp, Artificial sequence; identical to SEQ ID NO: 5
  Synthetic

SEQ ID NO: 8 - DNA, 30 bp, Artificial sequence; identical to SEQ ID NO: 4
  Synthetic

SEQ ID NO: 9 - DNA, 30 bp, Artificial sequence
  Synthetic
atttccgatttagaaacaagaagtggaaag

SEQ ID NO: 10 - DNA, 30 bp, Artificial sequence
  Synthetic
tttttagacctcgaaaaaggaagttaaaat

SEQ ID NO: 11 - DNA, 30 bp, Artificial sequence
  Synthetic
atttttgaactagaaaaagtaagtaaaaag

SEQ ID NO: 12 - DNA, 30 bp, Artificial sequence
  Synthetic
tttttggatcttgaaatagaaagtcaaaat

SEQ ID NO: 13 - DNA, 30 bp, Artificial sequence
  Synthetic
attttggatctagaaatagaaagtcaaaac

SEQ ID NO: 14 - DNA, 30 bp, Artificial sequence
  Synthetic
tttttcgacctcgaaatagtaagtgaaaag

SEQ ID NO: 15 - DNA, 30 bp, Artificial sequence
  Synthetic
atttttgatctagaaatagtaagtaaaaaa

SEQ ID NO: 16 - DNA, 30 bp, Artificial sequence
  Synthetic
gtttttgagctcgaaagagcaagttaaaat

SEQ ID NO: 17 - DNA, 30 bp, Artificial sequence
  Synthetic
gttttagagctagaaatagcaagttaaaat

SEQ ID NO: 18 - DNA, 30 bp, Artificial sequence
  Synthetic
gttttagtgctagaaatagctcgttaaaat

SEQ ID NO: 19 - DNA, 30 bp, Artificial sequence; identical to SEQ ID NO: 18
  Synthetic

SEQ ID NO: 20 - DNA, 30 bp, Artificial sequence
  Synthetic
gttttagggctagaaatagcgtgttaaaat

SEQ ID NO: 21 - DNA, 30 bp, Artificial sequence
  Synthetic
gttttagcgctagaaatagcatgttaaaat

SEQ ID NO: 22 - DNA, 30 bp, Artificial sequence
  Synthetic
gttttagagctagaaatagcgtgttaaaat

SEQ ID NO: 23 - DNA, 30 bp, Artificial sequence
  Synthetic
gttttagtgctagaaatagcaagttaaaat

SEQ ID NO: 24 - DNA, 30 bp, Artificial sequence
  Synthetic
gttttagggctagaaatagcatgttaaaat

SEQ ID NO: 25 - DNA, 30 bp, Artificial sequence; identical to SEQ ID NO: 21
  Synthetic

SEQ ID NO: 26 - DNA, 30 bp, Artificial sequence
  Synthetic
gttttagagctagaaatagctggttaaaat

SEQ ID NO: 27 - DNA, 30 bp, Artificial sequence
  Synthetic
gcgttatagctattcttagcaagttaacgt

SEQ ID NO: 28 - DNA, 30 bp, Artificial sequence
  Synthetic
ggattagagctagtcatagcaagttaatgt

SEQ ID NO: 29 - DNA, 30 bp, Artificial sequence
  Synthetic
gcattagagctacagatagcaagttaatat

SEQ ID NO: 30 - DNA, 30 bp, Artificial sequence
  Synthetic
gaattagagctagagatagcaagttaatct

SEQ ID NO: 31 - DNA, 30 bp, Artificial sequence
  Synthetic
gcattagagctacaggtagcaagttaatat

SEQ ID NO: 32 - DNA, 30 bp, Artificial sequence
  Synthetic
gaattatagctatagttagcaagttaattt

SEQ ID NO: 33 - DNA, 30 bp, Artificial sequence
  Synthetic
gcattagagctactagtagcaagttaattt

SEQ ID NO: 34 - DNA, 30 bp, Artificial sequence
  Synthetic
ggtttacagctaattgtagcaagttaaagt

SEQ ID NO: 35 - DNA, 30 bp, Artificial sequence
  Synthetic
ggtttagagctaaagatagcaagttaaaat

SEQ ID NO: 36 - DNA, 30 bp, Artificial sequence
  Synthetic
gaattatagctaagggtagcaagttaatat

SEQ ID NO: 37 - DNA, 30 bp, Artificial sequence
  Synthetic
gcatgagagctagaaatagcaagttcgtgt

SEQ ID NO: 38 - DNA, 30 bp, Artificial sequence
  Synthetic
ggtatagagctagaaatagcaagttttact

SEQ ID NO: 39 - DNA, 30 bp, Artificial sequence; identical to SEQ ID NO: 17
  Synthetic

SEQ ID NO: 40 - DNA, 30 bp, Artificial sequence; identical to SEQ ID NO: 17
  Synthetic

SEQ ID NO: 41 - DNA, 30 bp, Artificial sequence
  Synthetic
gcttcggagctagaaatagcaagtcgaaat

SEQ ID NO: 42 - DNA, 30 bp, Artificial sequence
  Synthetic
gcttttaagctagaaatagcaagtagaagt

SEQ ID NO: 43 - DNA, 30 bp, Artificial sequence
  Synthetic
gttggtgagttagaaataacaagtaccaat

SEQ ID NO: 44 - DNA, 30 bp, Artificial sequence
  Synthetic
  misc_feature (1)..(1): wherein N at position (1) to (1) is defined as any nucleotide
  misc_feature (5)..(6): wherein N at positions (5) to (6) are defined as any nucleotide
  misc_feature (9)..(12): wherein N at positions (9) to (12) are defined as any nucleotide
  misc_feature (17)..(20): wherein N at positions (17) to (20) are defined as any nucleotide
  misc_feature (25)..(26): wherein N at positions (25) to (26) are defined as any nucleotide
  misc_feature (30)..(30): wherein N at positions (30) to (30) are defined as any nucleotide
ntttnngannnngaaannnnaagtnnaaan

SEQ ID NO: 45 - DNA, 30 bp, Artificial sequence
  Synthetic
  misc_feature (1)..(1): wherein N at position (1) to (1) is defined as any nucleotide
  misc_feature (6)..(6): wherein N at position (6) to (6) is defined as any nucleotide
  misc_feature (9)..(9): wherein N at position (9) to (9) is defined as any nucleotide
  misc_feature (12)..(12): wherein N at position (12) to (12) is defined as any nucleotide
  misc_feature (17)..(17): wherein N at position (17) to (17) is defined as any nucleotide
  misc_feature (20)..(20): wherein N at position (20) to (20) is defined as any nucleotide
  misc_feature (25)..(25): wherein N at position (25) to (25) is defined as any nucleotide
  misc_feature (30)..(30): wherein N at position (30) to (30) is defined as any nucleotide
nttttnganctngaaanagnaagtnaaaan

SEQ ID NO: 46 - DNA, 30 bp, Artificial sequence
  Synthetic
  misc_feature (8)..(8): wherein N at position (8) to (8) is defined as any nucleotide
  misc_feature (21)..(23): wherein N at positions (21) to (23) are defined as any nucleotide
gttttagngctagaaatagcnnnttaaaat

SEQ ID NO: 47 - DNA, 30 bp, Artificial sequence
  Synthetic
  misc_feature (2)..(3): wherein N at positions (2) to (3) are defined as any nucleotide
  misc_feature (7)..(7): wherein N at position (7) to (7) is defined as any nucleotide
  misc_feature (13)..(16): wherein N at positions (13) to (16) are defined as any nucleotide
  misc_feature (24)..(24): wherein N at position (24) to (24) is defined as any nucleotide
  misc_feature (28)..(29): wherein N at positions (28) to (29) are defined as any nucleotide
gnnttanagctannnntagcaagntaannt

SEQ ID NO: 48 - DNA, 30 bp, Artificial sequence
  Synthetic
  misc_feature (2)..(7): wherein N at positions (2) to (7) are defined as any nucleotide
  misc_feature (24)..(29): wherein N at positions (24) to (29) are defined as any nucleotide
gnnnnnnagctagaaatagcaagnnnnnnt

SEQ ID NO: 49 - DNA, 30 bp, Artificial sequence
  Synthetic
  misc_feature (2)..(5): wherein N at positions (2) to (5) are defined as any nucleotide
  misc_feature (10)..(12): wherein N at positions (10) to (12) are defined as any nucleotide
  misc_feature (17)..(19): wherein N at positions (17) to (19) are defined as any nucleotide
  misc_feature (26)..(29): wherein N at positions (26) to (29) are defined as any nucleotide
gnnnntgagnnngaaannncaagtannnnt